European Patent Specification EP 3 572 427 B1, published June 25, 2025. Title: BCMA-TARGETING ANTIBODY AND USE THEREOF. Applicant: CARSGEN THERAPEUTICS CO., LTD. Application PCT/CN2018/073863. The sequence listing filed with the application follows.

SEQUENCE LISTING (87 sequences)

SEQ ID NO: 1 - protein, 5 aa, Artificial sequence
  7A12, 7G2, 23F10 HCDR1
SYAMS

SEQ ID NO: 2 - protein, 17 aa, Artificial sequence
  7A12, 7G2, 23F10 HCDR1
AISGSGGSTYYADSVKG

SEQ ID NO: 3 - protein, 8 aa, Artificial sequence
  7A12 HCDR3
YPYLAFDY

SEQ ID NO: 4 - protein, 9 aa, Artificial sequence
  7G2 HCDR3
LSGDAAMDY

SEQ ID NO: 5 - protein, 10 aa, Artificial sequence
  23F10 HCDR3
VRPFWGTFDY

SEQ ID NO: 6 - protein, 12 aa, Artificial sequence
  7A12, 7G2, 23F10 LCDR1
RASQSVSSSYLA

SEQ ID NO: 7 - protein, 7 aa, Artificial sequence
  7A12, 7G2, 23F10 LCDR2
GASSRAT

SEQ ID NO: 8 - protein, 9 aa, Artificial sequence
  7A12 LCDR3
QQYGYPPSY

SEQ ID NO: 9 - protein, 9 aa, Artificial sequence
  7G2 LCDR3
QQYGYPPRY

SEQ ID NO: 10 - protein, 9 aa, Artificial sequence
  23F10 LCDR3
QQYFNPPEY

SEQ ID NO: 11 - protein, 109 aa, Artificial sequence
  Amino acid sequence of 7A12 light chain variable regoin
EIVLTQSPGTLSLSPGERATLSCRASQSVSSSYLAWYQQKPGQAPRLLIYGASSRATGIPDRFSGSGSGTDFTLTISRLEPEDFAVYYCQQYGYPPSYTFGQGTKVEIK

SEQ ID NO: 12 - DNA, 327 bp, Artificial sequence
  Nucleotide sequence of 7A12 light chain variable region
gaaatcgtgttaacgcagtctccaggcaccctgtctttgtctccaggggaaagagccaccctctcttgcagggccagtcagagtgttagcagcagctacttagcctggtaccagcagaaacctggccaggctcccaggctcctcatctatggagcatccagcagggccactggcatcccagacaggttcagtggcagtggatccgggacagacttcactctcaccatcagcagactggagcctgaagattttgcagtgtattactgtcagcagtacggttacccaccatcttacacgttcggccaggggaccaaagtggaaatcaaa

SEQ ID NO: 13 - protein, 117 aa, Artificial sequence
  Amino acid sequence of 7A12 heavy chain variable region
EVQLLESGGGLVQPGGSLRLSCAASGFTFSSYAMSWVRQAPGKGLEWVSAISGSGGSTYYADSVKGRFTISRDNSKNTLYLQMNSLRAEDTAVYYCARYPYLAFDYWGQGTLVTVSS

SEQ ID NO: 14 - DNA, 351 bp, Artificial sequence
  Nucleotide sequence of 7A12 heavy chain variable region
gaggtgcaattgctggagtctgggggaggcttggtacagcctggggggtccctgagactctcctgtgcagcctccggattcacctttagcagttatgccatgagctgggtccgccaggctccagggaaggggctggagtgggtctcagctattagtggtagtggtggtagcacatactacgcagactccgtgaagggccggttcaccatctccagagacaattccaagaacacgctgtatctgcagatgaacagcctgagagccgaggacacggccgtatattactgtgcgcgttacccatacctggcattcgactactggggccaaggaaccctggtcaccgtctcgagt

SEQ ID NO: 15 - protein, 109 aa, Artificial sequence
  Amino acid sequence of 7G2 light chain variable region
EIVLTQSPGTLSLSPGERATLSCRASQSVSSSYLAWYQQKPGQAPRLLIYGASSRATGIPDRFSGSGSGTDFTLTISRLEPEDFAVYYCQQYGYPPRYTFGQGTKVEIK

SEQ ID NO: 16 - DNA, 327 bp, Artificial sequence
  Nucleotide sequence of 7G2 light variable region
gaaatcgtgttaacgcagtctccaggcaccctgtctttgtctccaggggaaagagccaccctctcttgcagggccagtcagagtgttagcagcagctacttagcctggtaccagcagaaacctggccaggctcccaggctcctcatctatggagcatccagcagggccactggcatcccagacaggttcagtggcagtggatccgggacagacttcactctcaccatcagcagactggagcctgaagattttgcagtgtattactgtcagcagtacggttacccaccaagatacacgttcggccaggggaccaaagtggaaatcaaa

SEQ ID NO: 17 - protein, 118 aa, Artificial sequence
  Amino acid sequence of 7G2 heavy chain variable region
EVQLLESGGGLVQPGGSLRLSCAASGFTFSSYAMSWVRQAPGKGLEWVSAISGSGGSTYYADSVKGRFTISRDNSKNTLYLQMNSLRAEDTAVYYCAKLSGDAAMDYWGQGTLVTVSS

SEQ ID NO: 18 - DNA, 354 bp, Artificial sequence
  Nucleotide sequence of 7G2 heavy chain variable region
gaggtgcaattgctggagtctgggggaggcttggtacagcctggggggtccctgagactctcctgtgcagcctccggattcacctttagcagttatgccatgagctgggtccgccaggctccagggaaggggctggagtgggtctcagctattagtggtagtggtggtagcacatactacgcagactccgtgaagggccggttcaccatctccagagacaattccaagaacacgctgtatctgcagatgaacagcctgagagccgaggacacggccgtatattactgtgcgaaactgtctggtgatgcagcaatggactactggggccaaggaaccctggtcaccgtctcgagt

SEQ ID NO: 19 - protein, 109 aa, Artificial sequence
  Amino acid sequence of 23F10 light chain variable region
EIVLTQSPGTLSLSPGERATLSCRASQSVSSSYLAWYQQKPGQAPRLLIYGASSRATGIPDRFSGSGSGTDFTLTISRLEPEDFAVYYCQQYFNPPEYTFGQGTKVEIK

SEQ ID NO: 20 - DNA, 327 bp, Artificial sequence
  Nucleotide sequence of 23F10 light chain variable region
gaaatcgtgttaacgcagtctccaggcaccctgtctttgtctccaggggaaagagccaccctctcttgcagggccagtcagagtgttagcagcagctacttagcctggtaccagcagaaacctggccaggctcccaggctcctcatctatggagcatccagcagggccactggcatcccagacaggttcagtggcagtggatccgggacagacttcactctcaccatcagcagactggagcctgaagattttgcagtgtattactgtcagcagtacttcaacccaccagaatacacgttcggccaggggaccaaagtggaaatcaaa

SEQ ID NO: 21 - protein, 119 aa, Artificial sequence
  Amino acid sequence of 23F10 heavy chain variable region
EVQLLESGGGLVQPGGSLRLSCAASGFTFSSYAMSWVRQAPGKGLEWVSAISGSGGSTYYADSVKGRFTISRDNSKNTLYLQMNSLRAEDTAVYYCAKVRPFWGTFDYWGQGTLVTVSS

SEQ ID NO: 22 - DNA, 357 bp, Artificial sequence
  Nucleotide sequence of 23F10 heavy chain variable region
gaggtgcaattgctggagtctgggggaggcttggtacagcctggggggtccctgagactctcctgtgcagcctccggattcacctttagcagttatgccatgagctgggtccgccaggctccagggaaggggctggagtgggtctcagctattagtggtagtggtggtagcacatactacgcagactccgtgaagggccggttcaccatctccagagacaattccaagaacacgctgtatctgcagatgaacagcctgagagccgaggacacggccgtatattactgtgcgaaagttcgtccattctggggtactttcgactactggggccaaggaaccctggtcaccgtctcgagt

SEQ ID NO: 23 - protein, 21 aa, Artificial sequence
  Amino acid sequence of CD8alpha signal peptide
MALPVTALLLPLALLLHAARP

SEQ ID NO: 24 - DNA, 63 bp, Artificial sequence
  Nucleotide sequence of CD8alpha signal peptide
atggccttaccagtgaccgccttgctcctgccgctggccttgctgctccacgccgccaggccg

SEQ ID NO: 25 - protein, 45 aa, Artificial sequence
  Amino acid sequence of CD8 hinge
TTTPAPRPPTPAPTIASQPLSLRPEACRPAAGGAVHTRGLDFACD

SEQ ID NO: 26 - DNA, 135 bp, Artificial sequence
  Nucleotide sequence of CD8 hinge
accacgacgccagcgccgcgaccaccaacaccggcgcccaccatcgcgtcgcagcccctgtccctgcgcccagaggcgtgccggccagcggcggggggcgcagtgcacacgagggggctggacttcgcctgtgat

SEQ ID NO: 27 - protein, 27 aa, Artificial sequence
  Amino acid sequence of CD28 transmembrane region
FWVLVVVGGVLACYSLLVTVAFIIFWV

SEQ ID NO: 28 - DNA, 81 bp, Artificial sequence
  Nucleotide sequence of CD28 transmembrane region
ttttgggtgctggtggtggttggtggagtcctggcttgctatagcttgctagtaacagtggcctttattattttctgggtg

SEQ ID NO: 29 - protein, 41 aa, Artificial sequence
  Amino acid sequence of CD28 intracellular region
RSKRSRLLHSDYMNMTPRRPGPTRKHYQPYAPPRDFAAYRS

SEQ ID NO: 30 - DNA, 123 bp, Artificial sequence
  Nucleotide sequence of CD28 intracellular region
aggagtaagaggagcaggctcctgcacagtgactacatgaacatgactccccgccgccccgggccaacccgcaagcattaccagccctatgccccaccacgcgacttcgcagcctatcgctcc

SEQ ID NO: 31 - protein, 113 aa, Artificial sequence
  Amino acid sequence of CD3Z domain
RVKFSRSADAPAYQQGQNQLYNELNLGRREEYDVLDKRRGRDPEMGGKPQRRKNPQEGLYNELQKDKMAEAYSEIGMKGERRRGKGHDGLYQGLSTATKDTYDALHMQALPPR

SEQ ID NO: 32 - DNA, 339 bp, Artificial sequence
  Nucleotide sequence of CD3Z domain
agagtgaagttcagcaggagcgcagacgcccccgcgtaccagcagggccagaaccagctctataacgagctcaatctaggacgaagagaggagtacgatgttttggacaagagacgtggccgggaccctgagatggggggaaagccgcagagaaggaagaaccctcaggaaggcctgtacaatgaactgcagaaagataagatggcggaggcctacagtgagattgggatgaaaggcgagcgccggaggggcaaggggcacgatggcctttaccagggtctcagtacagccaccaaggacacctacgacgcccttcacatgcaggccctgccccctcgc

SEQ ID NO: 33 - protein, 21 aa, Artificial sequence
  Amino acid sequence of CD8 transmembrane region
IYIWAPLAGTCGVLLLSLVIT

SEQ ID NO: 34 - DNA, 63 bp, Artificial sequence
  Nucleotide sequence of CD8 transmembrane region
atctacatctgggcgcccttggccgggacttgtggggtccttctcctgtcactggttatcacc

SEQ ID NO: 35 - protein, 42 aa, Artificial sequence
  Amino acid sequence of CD137 intracellular region
KRGRKKLLYIFKQPFMRPVQTTQEEDGCSCRFPEEEEGGCEL

SEQ ID NO: 36 - DNA, 126 bp, Artificial sequence
  Nucleotide sequence of CD137 intracellular region
aaacggggcagaaagaaactcctgtatatattcaaacaaccatttatgagaccagtacaaactactcaagaggaagatggctgtagctgccgatttccagaagaagaagaaggaggatgtgaactg

SEQ ID NO: 37 - protein, 184 aa, Artificial sequence
  BCMA amino acid sequence
MLQMAGQCSQNEYFDSLLHACIPCQLRCSSNTPPLTCQRYCNASVTNSVKGTNAILWTCLGLSLIISLAVFVLMFLLRKINSEPLKDEFKNTGSGLLGMANIDLEKSRTGDEIILPRGLEYTVEECTCEDCIKSKPKVDSDHCFPLPAMEEGATILVTTKTNDYCKSLPAALSATEIEKSISAR

SEQ ID NO: 38 - protein, 54 aa, Artificial sequence
  Human BCMA extracellular segment Met1-Ala54
MLQMAGQCSQNEYFDSLLHACIPCQLRCSSNTPPLTCQRYCNASVTNSVKGTNA

SEQ ID NO: 39 - DNA, 162 bp, Artificial sequence
  Nucleotide sequence of human BCMA extracellular segment Met1-Ala54
atgctgcagatggccggccagtgcagccagaacgagtacttcgacagcctgctgcacgcctgcatcccctgccagctgcggtgcagcagcaacaccccccccctgacctgccagcggtactgcaacgccagcgtgaccaacagcgtgaagggcaccaacgcc

SEQ ID NO: 40 - protein, 283 aa, Artificial sequence
  BCMA_huFc
MLQMAGQCSQNEYFDSLLHACIPCQLRCSSNTPPLTCQRYCNASVTNSVKGTNAGSDKTHTCPPCPAPELLGGPSVFLFPPKPKDTLMISRTPEVTCVVVDVSHEDPEVKFNWYVDGVEVHNAKTKPREEQYNSTYRVVSVLTVLHQDWLNGKEYKCKVSNKALPAPIEKTISKAKGQPREPQVYTLPPSRDELTKNQVSLWCLVKGFYPSDIAVEWESNGQPENNYKTTPPVLDSDGSFFLYSKLTVDKSRWQQGNVFSCSVMHEALHNHYTQKSLSLSPGK

SEQ ID NO: 41 - DNA, 849 bp, Artificial sequence
  Nucleotide sequence of BCMA_huFc
atgctgcagatggccggccagtgcagccagaacgagtacttcgacagcctgctgcacgcctgcatcccctgccagctgcggtgcagcagcaacaccccccccctgacctgccagcggtactgcaacgccagcgtgaccaacagcgtgaagggcaccaacgccggatccgacaaaactcacacatgcccaccgtgcccagcacctgaactcctggggggaccgtcagtcttcctcttccccccaaaacccaaggacaccctcatgatctcccggacccctgaggtcacatgcgtggtggtggacgtgagccacgaagaccctgaggtcaagttcaactggtacgtggacggcgtggaggtgcataatgccaagacaaagccgcgggaggagcagtacaacagcacgtaccgtgtggtcagcgtcctcaccgtcctgcaccaggactggctgaatggcaaggagtacaagtgcaaggtctccaacaaagccctcccagcccccatcgagaaaaccatctccaaagccaaagggcagccccgagaaccacaggtgtacaccctgcccccatcccgggatgagctgaccaagaaccaggtcagcctgtggtgcctggtcaaaggcttctatcccagcgacatcgccgtggagtgggagagcaatgggcagccggagaacaactacaagaccacgcctcccgtgctggactccgacggctccttcttcctctatagcaagctcaccgtggacaagagcaggtggcagcaggggaacgtcttctcatgctccgtgatgcatgaggctctgcacaaccactacacgcagaagagcctctccctgtctccgggtaaa

SEQ ID NO: 42 - protein, 281 aa, Artificial sequence
  BCMA_muFc
MLQMAGQCSQNEYFDSLLHACIPCQLRCSSNTPPLTCQRYCNASVTNSVKGTNAGSRDCGCKPCICTVPEVSSVFIFPPKPKDVLTITLTPKVTCVVVDISKDDPEVQFSWFVDDVEVHTAQTQPREEQFNSTFRSVSELPIMHQDWLNGKEFKCRVNSAAFPAPIEKTISKTKGRPKAPQVYTIPPPKEQMAKDKVSLTCMITDFFPEDITVEWQWNGQPAENYKNTQPIMDTDGSYFVYSKLNVQKSNWEAGNTFTCSVLHEGLHNHHTEKSLSHSPGK

SEQ ID NO: 43 - DNA, 843 bp, Artificial sequence
  Nucleotide sequence of BCMA_muFc
atgctgcagatggccggccagtgcagccagaacgagtacttcgacagcctgctgcacgcctgcatcccctgccagctgcggtgcagcagcaacaccccccccctgacctgccagcggtactgcaacgccagcgtgaccaacagcgtgaagggcaccaacgccggatccagggattgtggttgtaagccttgcatatgtacagtcccagaagtatcatctgtcttcatcttccccccaaagcccaaggatgtgctcaccattactctgactcctaaggtcacgtgtgttgtggtagacatcagcaaggatgatcccgaggtccagttcagctggtttgtagatgatgtggaggtgcacacagctcagacgcaaccccgggaggagcagttcaacagcactttccgctcagtcagtgaacttcccatcatgcaccaggactggctcaatggcaaggagttcaaatgcagggtcaacagtgcagctttccctgcccccatcgagaaaaccatctccaaaaccaaaggcagaccgaaggctccacaggtgtacaccattccacctcccaaggagcagatggccaaggataaagtcagtctgacctgcatgataacagacttcttccctgaagacattactgtggagtggcagtggaatgggcagccagcggagaactacaagaacactcagcccatcatggacacagatggctcttacttcgtctacagcaagctcaatgtgcagaagagcaactgggaggcaggaaatactttcacctgctctgtgttacatgagggcctgcacaaccaccatactgagaagagcctctcccactctcctggtaaa

SEQ ID NO: 44 - DNA, 589 bp, Artificial sequence
  Nucleotide sequence of human BCMA with introduced restriction sites MluI, SalI
acgcgtcctagcgctaccggtcgccaccatgttgcagatggctgggcagtgctcccaaaatgaatattttgacagtttgttgcatgcttgcataccttgtcaacttcgatgttcttctaatactcctcctctaacatgtcagcgttattgtaatgcaagtgtgaccaattcagtgaaaggaacgaatgcgattctctggacctgtttgggactgagcttaataatttctttggcagttttcgtgctaatgtttttgctaaggaagataaactctgaaccattaaaggacgagtttaaaaacacaggatcaggtctcctgggcatggctaacattgacctggaaaagagcaggactggtgatgaaattattcttccgagaggcctcgagtacacggtggaagaatgcacctgtgaagactgcatcaagagcaaaccgaaggtcgactctgaccattgctttccactcccagctatggaggaaggcgcaaccattcttgtcaccacgaaaacgaatgactattgcaagagcctgccagctgctttgagtgctacggagatagagaaatcaatttctgctaggtaagtcgac

SEQ ID NO: 45 - protein, 365 aa, Artificial sequence
  APRIL_huFc
HSVLHLVPINATSKDDSDVTEVMWQPALRRGRGLQAQGYGVRIQDAGVYLLYSQVLFQDVTFTMGQVVSREGQGRQETLFRCIRSMPSHPDRAYNSCYSAGVFHLHQGDILSVIIPRARAKLNLSPHGTFLGFVKLGSDKTHTCPPCPAPELLGGPSVFLFPPKPKDTLMISRTPEVTCVVVDVSHEDPEVKFNWYVDGVEVHNAKTKPREEQYNSTYRVVSVLTVLHQDWLNGKEYKCKVSNKALPAPIEKTISKAKGQPREPQVYTLPPSRDELTKNQVSLWCLVKGFYPSDIAVEWESNGQPENNYKTTPPVLDSDGSFFLYSKLTVDKSRWQQGNVFSCSVMHEALHNHYTQKSLSLSPGK

SEQ ID NO: 46 - DNA, 1095 bp, Artificial sequence
  Nucleotide sequence of APRIL_huFc
cacagcgtgctgcacctggtgcccatcaacgccaccagcaaggacgacagcgacgtgaccgaggtgatgtggcagcccgccctgcggcggggccggggcctgcaggcccagggctacggcgtgcggatccaggacgccggcgtgtacctgctgtacagccaggtgctgttccaggacgtgaccttcaccatgggccaggtggtgagccgggagggccagggccggcaggagaccctgttccggtgcatccggagcatgcccagccaccccgaccgggcctacaacagctgctacagcgccggcgtgttccacctgcaccagggcgacatcctgagcgtgatcatcccccgggcccgggccaagctgaacctgagcccccacggcaccttcctgggcttcgtgaagctgggatccgacaaaactcacacatgcccaccgtgcccagcacctgaactcctggggggaccgtcagtcttcctcttccccccaaaacccaaggacaccctcatgatctcccggacccctgaggtcacatgcgtggtggtggacgtgagccacgaagaccctgaggtcaagttcaactggtacgtggacggcgtggaggtgcataatgccaagacaaagccgcgggaggagcagtacaacagcacgtaccgtgtggtcagcgtcctcaccgtcctgcaccaggactggctgaatggcaaggagtacaagtgcaaggtctccaacaaagccctcccagcccccatcgagaaaaccatctccaaagccaaagggcagccccgagaaccacaggtgtacaccctgcccccatcccgggatgagctgaccaagaaccaggtcagcctgtggtgcctggtcaaaggcttctatcccagcgacatcgccgtggagtgggagagcaatgggcagccggagaacaactacaagaccacgcctcccgtgctggactccgacggctccttcttcctctatagcaagctcaccgtggacaagagcaggtggcagcaggggaacgtcttctcatgctccgtgatgcatgaggctctgcacaaccactacacgcagaagagcctctccctgtctccgggtaaa

SEQ ID NO: 47 - protein, 242 aa, Artificial sequence
  47 7A12 scFv
EVQLLESGGGLVQPGGSLRLSCAASGFTFSSYAMSWVRQAPGKGLEWVSAISGSGGSTYYADSVKGRFTISRDNSKNTLYLQMNSLRAEDTAVYYCARYPYLAFDYWGQGTLVTVSSGGGGSGGGGSGGGGSEIVLTQSPGTLSLSPGERATLSCRASQSVSSSYLAWYQQKPGQAPRLLIYGASSRATGIPDRFSGSGSGTDFTLTISRLEPEDFAVYYCQQYGYPPSYTFGQGTKVEIKR

SEQ ID NO: 48 - protein, 243 aa, Artificial sequence
  7G2 scFv
EVQLLESGGGLVQPGGSLRLSCAASGFTFSSYAMSWVRQAPGKGLEWVSAISGSGGSTYYADSVKGRFTISRDNSKNTLYLQMNSLRAEDTAVYYCAKLSGDAAMDYWGQGTLVTVSSGGGGSGGGGSGGGGSEIVLTQSPGTLSLSPGERATLSCRASQSVSSSYLAWYQQKPGQAPRLLIYGASSRATGIPDRFSGSGSGTDFTLTISRLEPEDFAVYYCQQYGYPPRYTFGQGTKVEIKR

SEQ ID NO: 49 - DNA, 26 bp, Artificial sequence
  Primer LMF
caggaaacagctatgaccatgattac

SEQ ID NO: 50 - DNA, 80 bp, Artificial sequence
  Primer BH1R
  misc_feature (44)..(45): n is a, c, g, or t
  misc_feature (47)..(48): n is a, c, g, or t
  misc_feature (50)..(51): n is a, c, g, or t
  misc_feature (53)..(54): n is a, c, g, or t
  misc_feature (56)..(57): n is a, c, g, or t
  misc_feature (59)..(60): n is a, c, g, or t
tgagacccactccagccccttccctggagcctggcggacccamnnmnnmnnmnnmnnmnnaaaggtgaatccggaggctg

SEQ ID NO: 51 - DNA, 67 bp, Artificial sequence
  Primer BH2F
  misc_feature (18)..(19): n is a, c, g, or t
  misc_feature (24)..(25): n is a, c, g, or t
  misc_feature (27)..(28): n is a, c, g, or t
  misc_feature (30)..(31): n is a, c, g, or t
  misc_feature (33)..(34): n is a, c, g, or t
  misc_feature (39)..(40): n is a, c, g, or t
  misc_feature (45)..(46): n is a, c, g, or t
ggctggagtgggtctcannkattnnknnknnknnkggtnnkacannktacgcagactccgtgaaggg

SEQ ID NO: 52 - DNA, 30 bp, Artificial sequence
  Primer FdR
gacgttagtaaatgaattttctgtatgagg

SEQ ID NO: 53 - DNA, 85 bp, Artificial sequence
  Primer BL1R
  misc_feature (44)..(45): n is a, c, g, or t
  misc_feature (50)..(51): n is a, c, g, or t
  misc_feature (53)..(54): n is a, c, g, or t
  misc_feature (56)..(57): n is a, c, g, or t
  misc_feature (59)..(60): n is a, c, g, or t
  misc_feature (62)..(63): n is a, c, g, or t
  misc_feature (65)..(66): n is a, c, g, or t
gatgaggagcctgggagcctggccaggtttctgctggtaccamnntaamnnmnnmnnmnnmnnmnnctgactggccctgcaagag

SEQ ID NO: 54 - DNA, 58 bp, Artificial sequence
  Primer BL2F
  misc_feature (23)..(24): n is a, c, g, or t
  misc_feature (26)..(27): n is a, c, g, or t
  misc_feature (29)..(30): n is a, c, g, or t
  misc_feature (32)..(33): n is a, c, g, or t
  misc_feature (35)..(36): n is a, c, g, or t
ccaggctcccaggctcctcatcnnknnknnknnknnkagggccactggcatcccagac

SEQ ID NO: 55 - protein, 244 aa, Artificial sequence
  23F10 scFv
EVQLLESGGGLVQPGGSLRLSCAASGFTFSSYAMSWVRQAPGKGLEWVSAISGSGGSTYYADSVKGRFTISRDNSKNTLYLQMNSLRAEDTAVYYCAKVRPFWGTFDYWGQGTLVTVSSGGGGSGGGGSGGGGSEIVLTQSPGTLSLSPGERATLSCRASQSVSSSYLAWYQQKPGQAPRLLIYGASSRATGIPDRFSGSGSGTDFTLTISRLEPEDFAVYYCQQYFNPPEYTFGQGTKVEIKR

SEQ ID NO: 56 - protein, 119 aa, Artificial sequence
  25C2 VH(AA)
EVQLLESGGGLVQPGGSLRLSCAASGFTFGGNAMSWVRQAPGKGLEWVSAISGNGGSTFYADSVKGRFTISRDNSKNTLYLQMNSLRAEDTAVYYCAKVRPFWGTFDYWGQGTLVTVSS

SEQ ID NO: 57 - DNA, 357 bp, Artificial sequence
  25C2 VH
gaggtgcaattgctggagtctgggggaggcttggtacagcctggggggtccctgagactctcctgtgcagcctccggattcacctttggcggtaatgccatgtcctgggtccgccaggctccagggaaggggctggagtgggtctcagcaattagtggtaatggtggtagtacattctacgcagactccgtgaagggccggttcaccatctccagagacaattccaagaacacgctgtatctgcagatgaacagcctgagagccgaggacacggccgtatattactgtgcgaaagttcgtccattctggggtactttcgactactggggccaaggaaccctggtcaccgtctcgagt

SEQ ID NO: 58 - protein, 119 aa, Artificial sequence
  25D2 VH(AA)
EVQLLESGGGLVQPGGSLRLSCAASGFTFRSYAMSWVRQAPGKGLEWVSAISGGGGNTFYADSVKGRFTISRDNSKNTLYLQMNSLRAEDTAVYYCAKVRPFWGTFDYWGQGTLVTVSS

SEQ ID NO: 59 - DNA, 357 bp, Artificial sequence
  25D2 VH
gaggtgcaattgctggagtctgggggaggcttggtacagcctggggggtccctgagactctcctgtgcagcctccggattcacctttaggagctatgccatgagctgggtccgccaggctccagggaaggggctggagtgggtctcagctattagtggcggtggtggtaacacattctacgcagactccgtgaagggccggttcaccatctccagagacaattccaagaacacgctgtatctgcagatgaacagcctgagagccgaggacacggccgtatattactgtgcgaaagttcgtccattctggggtactttcgactactggggccaaggaaccctggtcaccgtctcgagt

SEQ ID NO: 60 - protein, 5 aa, Artificial sequence
  25C2  HCDR1
GNAMS

SEQ ID NO: 61 - protein, 17 aa, Artificial sequence
  25C2  HCDR2
AISGNGGSTFYADSVKG

SEQ ID NO: 62 - protein, 5 aa, Artificial sequence
  25D2  HCDR1
SYAMS

SEQ ID NO: 63 - protein, 17 aa, Artificial sequence
  25D2  HCDR2
AISGGGGNTFYADSVKG

SEQ ID NO: 64 - DNA, 732 bp, Artificial sequence
  25C2 scFv
gaggtgcaattgctggagtctgggggaggcttggtacagcctggggggtccctgagactctcctgtgcagcctccggattcacctttggcggtaatgccatgtcctgggtccgccaggctccagggaaggggctggagtgggtctcagcaattagtggtaatggtggtagtacattctacgcagactccgtgaagggccggttcaccatctccagagacaattccaagaacacgctgtatctgcagatgaacagcctgagagccgaggacacggccgtatattactgtgcgaaagttcgtccattctggggtactttcgactactggggccaaggaaccctggtcaccgtctcgagtggtggaggcggttcaggcggaggtggttctggcggtggcggatcggaaatcgtgttaacgcagtctccaggcaccctgtctttgtctccaggggaaagagccaccctctcttgcagggccagtcagagtgttagcagcagctacttagcctggtaccagcagaaacctggccaggctcccaggctcctcatctatggagcatccagcagggccactggcatcccagacaggttcagtggcagtggatccgggacagacttcactctcaccatcagcagactggagcctgaagattttgcagtgtattactgtcagcagtacttcaacccaccagaatacacgttcggccaggggaccaaagtggaaatcaaacgt

SEQ ID NO: 65 - protein, 244 aa, Artificial sequence
  25C2 scFv(AA)
EVQLLESGGGLVQPGGSLRLSCAASGFTFGGNAMSWVRQAPGKGLEWVSAISGNGGSTFYADSVKGRFTISRDNSKNTLYLQMNSLRAEDTAVYYCAKVRPFWGTFDYWGQGTLVTVSSGGGGSGGGGSGGGGSEIVLTQSPGTLSLSPGERATLSCRASQSVSSSYLAWYQQKPGQAPRLLIYGASSRATGIPDRFSGSGSGTDFTLTISRLEPEDFAVYYCQQYFNPPEYTFGQGTKVEIKR

SEQ ID NO: 66 - DNA, 732 bp, Artificial sequence
  25D2 scFv
gaggtgcaattgctggagtctgggggaggcttggtacagcctggggggtccctgagactctcctgtgcagcctccggattcacctttaggagctatgccatgagctgggtccgccaggctccagggaaggggctggagtgggtctcagctattagtggcggtggtggtaacacattctacgcagactccgtgaagggccggttcaccatctccagagacaattccaagaacacgctgtatctgcagatgaacagcctgagagccgaggacacggccgtatattactgtgcgaaagttcgtccattctggggtactttcgactactggggccaaggaaccctggtcaccgtctcgagtggtggaggcggttcaggcggaggtggttctggcggtggcggatcggaaatcgtgttaacgcagtctccaggcaccctgtctttgtctccaggggaaagagccaccctctcttgcagggccagtcagagtgttagcagcagctacttagcctggtaccagcagaaacctggccaggctcccaggctcctcatctatggagcatccagcagggccactggcatcccagacaggttcagtggcagtggatccgggacagacttcactctcaccatcagcagactggagcctgaagattttgcagtgtattactgtcagcagtacttcaacccaccagaatacacgttcggccaggggaccaaagtggaaatcaaacgt

SEQ ID NO: 67 - protein, 244 aa, Artificial sequence
  25D2 scFv(AA)
EVQLLESGGGLVQPGGSLRLSCAASGFTFRSYAMSWVRQAPGKGLEWVSAISGGGGNTFYADSVKGRFTISRDNSKNTLYLQMNSLRAEDTAVYYCAKVRPFWGTFDYWGQGTLVTVSSGGGGSGGGGSGGGGSEIVLTQSPGTLSLSPGERATLSCRASQSVSSSYLAWYQQKPGQAPRLLIYGASSRATGIPDRFSGSGSGTDFTLTISRLEPEDFAVYYCQQYFNPPEYTFGQGTKVEIKR

SEQ ID NO: 68 - DNA, 60 bp, Artificial sequence
  PD-1 signal peptide sequence
atgcagatcccacaggcgccctggccagtcgtctgggcggtgctacaactgggctggcgg

SEQ ID NO: 69 - DNA, 450 bp, Artificial sequence
  PD-1 extracellular segment sequence
ccaggatggttcttagactccccagacaggccctggaacccccccaccttctccccagccctgctcgtggtgaccgaaggggacaacgccaccttcacctgcagcttctccaacacatcggagagcttcgtgctaaactggtaccgcatgagccccagcaaccagacggacaagctggccgccttccccgaggaccgcagccagcccggccaggactgccgcttccgtgtcacacaactgcccaacgggcgtgacttccacatgagcgtggtcagggcccggcgcaatgacagcggcacctacctctgtggggccatctccctggcccccaaggcgcagatcaaagagagcctgcgggcagagctcagggtgacagagagaagggcagaagtgcccacagcccaccccagcccctcacccaggccagccggccagttccaaaccctggtg

SEQ ID NO: 70 - DNA, 321 bp, Artificial sequence
  DNA sequence of CH3 domain
cccccatgcccaccatgcccagcacctgagttcctggggggaccatcagtcttcctgttccccccaaaacccaaggacactctcatgatctcccggacccctgaggtcacgtgcgtggtggtggacgtgagccaggaagaccccgaggtccagttcaactggtacgtggatggcgtggaggtgcataatgccaagacaaagccgcgggaggagcagttcaacagcacgtaccgtgtggtcagcgtcctcaccgtcctgcaccaggactggctgaacggcaaggagtacaagtgcaaggtctccaacaaaggcctcccgtcc

SEQ ID NO: 71 - DNA, 49 bp, Artificial sequence
  Primer
acgcgtcctagcgctaccggtcgccaccatgcagatcccacaggcgccc

SEQ ID NO: 72 - DNA, 41 bp, Artificial sequence
  Primer
ctctcggggctgcccaccatacaccagggtttggaactggc

SEQ ID NO: 73 - DNA, 27 bp, Artificial sequence
  Primer
tatggtgggcagccccgagagccacag

SEQ ID NO: 74 - DNA, 40 bp, Artificial sequence
  Primer
aaaattcaaagtctgtttcactttacccggagacagggag

SEQ ID NO: 75 - protein, 465 aa, Artificial sequence
  7A12-BBZ
EVQLLESGGGLVQPGGSLRLSCAASGFTFSSYAMSWVRQAPGKGLEWVSAISGSGGSTYYADSVKGRFTISRDNSKNTLYLQMNSLRAEDTAVYYCARYPYLAFDYWGQGTLVTVSSGGGGSGGGGSGGGGSEIVLTQSPGTLSLSPGERATLSCRASQSVSSSYLAWYQQKPGQAPRLLIYGASSRATGIPDRFSGSGSGTDFTLTISRLEPEDFAVYYCQQYGYPPSYTFGQGTKVEIKRTTTPAPRPPTPAPTIASQPLSLRPEACRPAAGGAVHTRGLDFACDIYIWAPLAGTCGVLLLSLVITLYCKRGRKKLLYIFKQPFMRPVQTTQEEDGCSCRFPEEEEGGCELRVKFSRSADAPAYKQGQNQLYNELNLGRREEYDVLDKRRGRDPEMGGKPRRKNPQEGLYNELQKDKMAEAYSEIGMKGERRRGKGHDGLYQGLSTATKDTYDALHMQALPPR

SEQ ID NO: 76 - protein, 467 aa, Artificial sequence
  25C2-BBZ
EVQLLESGGGLVQPGGSLRLSCAASGFTFGGNAMSWVRQAPGKGLEWVSAISGNGGSTFYADSVKGRFTISRDNSKNTLYLQMNSLRAEDTAVYYCAKVRPFWGTFDYWGQGTLVTVSSGGGGSGGGGSGGGGSEIVLTQSPGTLSLSPGERATLSCRASQSVSSSYLAWYQQKPGQAPRLLIYGASSRATGIPDRFSGSGSGTDFTLTISRLEPEDFAVYYCQQYFNPPEYTFGQGTKVEIKRTTTPAPRPPTPAPTIASQPLSLRPEACRPAAGGAVHTRGLDFACDIYIWAPLAGTCGVLLLSLVITLYCKRGRKKLLYIFKQPFMRPVQTTQEEDGCSCRFPEEEEGGCELRVKFSRSADAPAYKQGQNQLYNELNLGRREEYDVLDKRRGRDPEMGGKPRRKNPQEGLYNELQKDKMAEAYSEIGMKGERRRGKGHDGLYQGLSTATKDTYDALHMQALPPR

SEQ ID NO: 77 - protein, 467 aa, Artificial sequence
  25D2-BBZ
EVQLLESGGGLVQPGGSLRLSCAASGFTFRSYAMSWVRQAPGKGLEWVSAISGGGGNTFYADSVKGRFTISRDNSKNTLYLQMNSLRAEDTAVYYCAKVRPFWGTFDYWGQGTLVTVSSGGGGSGGGGSGGGGSEIVLTQSPGTLSLSPGERATLSCRASQSVSSSYLAWYQQKPGQAPRLLIYGASSRATGIPDRFSGSGSGTDFTLTISRLEPEDFAVYYCQQYFNPPEYTFGQGTKVEIKRTTTPAPRPPTPAPTIASQPLSLRPEACRPAAGGAVHTRGLDFACDIYIWAPLAGTCGVLLLSLVITLYCKRGRKKLLYIFKQPFMRPVQTTQEEDGCSCRFPEEEEGGCELRVKFSRSADAPAYKQGQNQLYNELNLGRREEYDVLDKRRGRDPEMGGKPRRKNPQEGLYNELQKDKMAEAYSEIGMKGERRRGKGHDGLYQGLSTATKDTYDALHMQALPPR

SEQ ID NO: 78 - protein, 466 aa, Artificial sequence
  7G2-BBZ
EVQLLESGGGLVQPGGSLRLSCAASGFTFSSYAMSWVRQAPGKGLEWVSAISGSGGSTYYADSVKGRFTISRDNSKNTLYLQMNSLRAEDTAVYYCAKLSGDAAMDYWGQGTLVTVSSGGGGSGGGGSGGGGSEIVLTQSPGTLSLSPGERATLSCRASQSVSSSYLAWYQQKPGQAPRLLIYGASSRATGIPDRFSGSGSGTDFTLTISRLEPEDFAVYYCQQYGYPPRYTFGQGTKVEIKRTTTPAPRPPTPAPTIASQPLSLRPEACRPAAGGAVHTRGLDFACDIYIWAPLAGTCGVLLLSLVITLYCKRGRKKLLYIFKQPFMRPVQTTQEEDGCSCRFPEEEEGGCELRVKFSRSADAPAYKQGQNQLYNELNLGRREEYDVLDKRRGRDPEMGGKPRRKNPQEGLYNELQKDKMAEAYSEIGMKGERRRGKGHDGLYQGLSTATKDTYDALHMQALPPR

SEQ ID NO: 79 - protein, 468 aa, Artificial sequence
  7A12-28Z
EVQLLESGGGLVQPGGSLRLSCAASGFTFSSYAMSWVRQAPGKGLEWVSAISGSGGSTYYADSVKGRFTISRDNSKNTLYLQMNSLRAEDTAVYYCARYPYLAFDYWGQGTLVTVSSGGGGSGGGGSGGGGSEIVLTQSPGTLSLSPGERATLSCRASQSVSSSYLAWYQQKPGQAPRLLIYGASSRATGIPDRFSGSGSGTDFTLTISRLEPEDFAVYYCQQYGYPPSYTFGQGTKVEIKRTTTPAPRPPTPAPTIASQPLSLRPEACRPAAGGAVHTRGLDFACDFWVLVVVGGVLACYSLLVTVAFIIFWVRSKRSRLLHSDYMNMTPRRPGPTRKHYQPYAPPRDFAAYRSRVKFSRSADAPAYQQGQNQLYNELNLGRREEYDVLDKRRGRDPEMGGKPQRRKNPQEGLYNELQKDKMAEAYSEIGMKGERRRGKGHDGLYQGLSTATKDTYDALHMQALPPR

SEQ ID NO: 80 - protein, 510 aa, Artificial sequence
  7A12-28BBZ
EVQLLESGGGLVQPGGSLRLSCAASGFTFSSYAMSWVRQAPGKGLEWVSAISGSGGSTYYADSVKGRFTISRDNSKNTLYLQMNSLRAEDTAVYYCARYPYLAFDYWGQGTLVTVSSGGGGSGGGGSGGGGSEIVLTQSPGTLSLSPGERATLSCRASQSVSSSYLAWYQQKPGQAPRLLIYGASSRATGIPDRFSGSGSGTDFTLTISRLEPEDFAVYYCQQYGYPPSYTFGQGTKVEIKRTTTPAPRPPTPAPTIASQPLSLRPEACRPAAGGAVHTRGLDFACDFWVLVVVGGVLACYSLLVTVAFIIFWVRSKRSRLLHSDYMNMTPRRPGPTRKHYQPYAPPRDFAAYRSKRGRKKLLYIFKQPFMRPVQTTQEEDGCSCRFPEEEEGGCELRVKFSRSADAPAYQQGQNQLYNELNLGRREEYDVLDKRRGRDPEMGGKPQRRKNPQEGLYNELQKDKMAEAYSEIGMKGERRRGKGHDGLYQGLSTATKDTYDALHMQALPPR

SEQ ID NO: 81 - protein, 469 aa, Artificial sequence
  7G2-28Z
EVQLLESGGGLVQPGGSLRLSCAASGFTFSSYAMSWVRQAPGKGLEWVSAISGSGGSTYYADSVKGRFTISRDNSKNTLYLQMNSLRAEDTAVYYCAKLSGDAAMDYWGQGTLVTVSSGGGGSGGGGSGGGGSEIVLTQSPGTLSLSPGERATLSCRASQSVSSSYLAWYQQKPGQAPRLLIYGASSRATGIPDRFSGSGSGTDFTLTISRLEPEDFAVYYCQQYGYPPRYTFGQGTKVEIKRTTTPAPRPPTPAPTIASQPLSLRPEACRPAAGGAVHTRGLDFACDFWVLVVVGGVLACYSLLVTVAFIIFWVRSKRSRLLHSDYMNMTPRRPGPTRKHYQPYAPPRDFAAYRSRVKFSRSADAPAYQQGQNQLYNELNLGRREEYDVLDKRRGRDPEMGGKPQRRKNPQEGLYNELQKDKMAEAYSEIGMKGERRRGKGHDGLYQGLSTATKDTYDALHMQALPPR

SEQ ID NO: 82 - protein, 511 aa, Artificial sequence
  7G2-28BBZ
EVQLLESGGGLVQPGGSLRLSCAASGFTFSSYAMSWVRQAPGKGLEWVSAISGSGGSTYYADSVKGRFTISRDNSKNTLYLQMNSLRAEDTAVYYCAKLSGDAAMDYWGQGTLVTVSSGGGGSGGGGSGGGGSEIVLTQSPGTLSLSPGERATLSCRASQSVSSSYLAWYQQKPGQAPRLLIYGASSRATGIPDRFSGSGSGTDFTLTISRLEPEDFAVYYCQQYGYPPRYTFGQGTKVEIKRTTTPAPRPPTPAPTIASQPLSLRPEACRPAAGGAVHTRGLDFACDFWVLVVVGGVLACYSLLVTVAFIIFWVRSKRSRLLHSDYMNMTPRRPGPTRKHYQPYAPPRDFAAYRSKRGRKKLLYIFKQPFMRPVQTTQEEDGCSCRFPEEEEGGCELRVKFSRSADAPAYQQGQNQLYNELNLGRREEYDVLDKRRGRDPEMGGKPQRRKNPQEGLYNELQKDKMAEAYSEIGMKGERRRGKGHDGLYQGLSTATKDTYDALHMQALPPR

SEQ ID NO: 83 - protein, 470 aa, Artificial sequence
  25C2-28Z
EVQLLESGGGLVQPGGSLRLSCAASGFTFSSYAMSWVRQAPGKGLEWVSAISGSGGSTYYADSVKGRFTISRDNSKNTLYLQMNSLRAEDTAVYYCAKVRPFWGTFDYWGQGTLVTVSSGGGGSGGGGSGGGGSEIVLTQSPGTLSLSPGERATLSCRASQSVSSSYLAWYQQKPGQAPRLLIYGASSRATGIPDRFSGSGSGTDFTLTISRLEPEDFAVYYCQQYFNPPEYTFGQGTKVEIKRTTTPAPRPPTPAPTIASQPLSLRPEACRPAAGGAVHTRGLDFACDFWVLVVVGGVLACYSLLVTVAFIIFWVRSKRSRLLHSDYMNMTPRRPGPTRKHYQPYAPPRDFAAYRSRVKFSRSADAPAYQQGQNQLYNELNLGRREEYDVLDKRRGRDPEMGGKPQRRKNPQEGLYNELQKDKMAEAYSEIGMKGERRRGKGHDGLYQGLSTATKDTYDALHMQALPPR

SEQ ID NO: 84 - protein, 512 aa, Artificial sequence
  25C2-28BBZ
EVQLLESGGGLVQPGGSLRLSCAASGFTFSSYAMSWVRQAPGKGLEWVSAISGSGGSTYYADSVKGRFTISRDNSKNTLYLQMNSLRAEDTAVYYCAKVRPFWGTFDYWGQGTLVTVSSGGGGSGGGGSGGGGSEIVLTQSPGTLSLSPGERATLSCRASQSVSSSYLAWYQQKPGQAPRLLIYGASSRATGIPDRFSGSGSGTDFTLTISRLEPEDFAVYYCQQYFNPPEYTFGQGTKVEIKRTTTPAPRPPTPAPTIASQPLSLRPEACRPAAGGAVHTRGLDFACDFWVLVVVGGVLACYSLLVTVAFIIFWVRSKRSRLLHSDYMNMTPRRPGPTRKHYQPYAPPRDFAAYRSKRGRKKLLYIFKQPFMRPVQTTQEEDGCSCRFPEEEEGGCELRVKFSRSADAPAYQQGQNQLYNELNLGRREEYDVLDKRRGRDPEMGGKPQRRKNPQEGLYNELQKDKMAEAYSEIGMKGERRRGKGHDGLYQGLSTATKDTYDALHMQALPPR

SEQ ID NO: 85 - protein, 470 aa, Artificial sequence
  25D2-28Z
EVQLLESGGGLVQPGGSLRLSCAASGFTFRSYAMSWVRQAPGKGLEWVSAISGGGGNTFYADSVKGRFTISRDNSKNTLYLQMNSLRAEDTAVYYCAKVRPFWGTFDYWGQGTLVTVSSGGGGSGGGGSGGGGSEIVLTQSPGTLSLSPGERATLSCRASQSVSSSYLAWYQQKPGQAPRLLIYGASSRATGIPDRFSGSGSGTDFTLTISRLEPEDFAVYYCQQYFNPPEYTFGQGTKVEIKRTTTPAPRPPTPAPTIASQPLSLRPEACRPAAGGAVHTRGLDFACDFWVLVVVGGVLACYSLLVTVAFIIFWVRSKRSRLLHSDYMNMTPRRPGPTRKHYQPYAPPRDFAAYRSRVKFSRSADAPAYQQGQNQLYNELNLGRREEYDVLDKRRGRDPEMGGKPQRRKNPQEGLYNELQKDKMAEAYSEIGMKGERRRGKGHDGLYQGLSTATKDTYDALHMQALPPR

SEQ ID NO: 86 - protein, 512 aa, Artificial sequence
  25D2-28BBZ
EVQLLESGGGLVQPGGSLRLSCAASGFTFRSYAMSWVRQAPGKGLEWVSAISGGGGNTFYADSVKGRFTISRDNSKNTLYLQMNSLRAEDTAVYYCAKVRPFWGTFDYWGQGTLVTVSSGGGGSGGGGSGGGGSEIVLTQSPGTLSLSPGERATLSCRASQSVSSSYLAWYQQKPGQAPRLLIYGASSRATGIPDRFSGSGSGTDFTLTISRLEPEDFAVYYCQQYFNPPEYTFGQGTKVEIKRTTTPAPRPPTPAPTIASQPLSLRPEACRPAAGGAVHTRGLDFACDFWVLVVVGGVLACYSLLVTVAFIIFWVRSKRSRLLHSDYMNMTPRRPGPTRKHYQPYAPPRDFAAYRSKRGRKKLLYIFKQPFMRPVQTTQEEDGCSCRFPEEEEGGCELRVKFSRSADAPAYQQGQNQLYNELNLGRREEYDVLDKRRGRDPEMGGKPQRRKNPQEGLYNELQKDKMAEAYSEIGMKGERRRGKGHDGLYQGLSTATKDTYDALHMQALPPR

SEQ ID NO: 87 - protein, 412 aa, Artificial sequence
  C11D5.3-BBZ
QIQLVQSGPELKKPGETVKISCKASGYTFTDYSINWVKRAPGKGLKWMGWINTETREPAYAYDFRGRFAFSLETSASTAYLQINNLKYEDTATYFCALDYSYAMDYWGQGTSVTVSSGGGGSGGGGSGGGGSDIVLTQSPPSLAMSLGKRATISCRASESVTILGSHLIHWYQQKPGQPPTLLIQLASNTTTPAPRPPTPAPTIASQPLSLRPEACRPAAGGAVHTRGLDFACDIYIWAPLAGTCGVLLLSLVITLYCKRGRKKLLYIFKQPFMRPVQTTQEEDGCSCRFPEEEEGGCELRVKFSRSADAPAYKQGQNQLYNELNLGRREEYDVLDKRRGRDPEMGGKPRRKNPQEGLYNELQKDKMAEAYSEIGMKGERRRGKGHDGLYQGLSTATKDTYDALHMQALPPR